European Patent Application EP 4 230 743 A1, published August 23, 2023. Title: A microorganism having enhanced L- glutamine productivity and a method for L-glutamine using the same. Applicant: CJ CheilJedang Corporation. The sequence listing filed with the application follows.

SEQUENCE LISTING (12 sequences)

SEQ ID NO: 1 - protein, 610 aa, Unknown
  Phosphoenolpyruvate carboxykinase AA
MTTAAIRGLQGEAPTKNKELLNWIADAVELFQPEAVVFVDGSQAEWDRMAEDLVEAGTLIKLNEEKRPNSYLARSNPSDVARVESRTFICSEKEEDAGPTNNWAPPQAMKDEMSKHYAGSMKGRTMYVVPFCMGPISDPDPKLGVQLTDSEYVVMSMRIMTRMGIEALDKIGANGSFVRCLHSVGAPLEPGQEDVAWPCNDTKYITQFPETKEIWSYGSGYGGNAILAKKCYALRIASVMAREEGWMAEHMLILKLINPEGKAYHIAAAFPSACGKTNLAMITPTIPGWTAQVVGDDIAWLKLREDGLYAVNPENGFFGVAPGTNYASNPIAMKTMEPGNTLFTNVALTDDGDIWWEGMDGDAPAHLIDWMGNDWTPESDENAAHPNSRYCVAIDQSPAAAPEFNDWEGVKIDAILFGGRRADTVPLVTQTYDWEHGTMVGALLASGQTAASAEAKVGTLRHDPMAMLPFIGYNAGEYLQNWIDMGNKGGDKMPSIFLVNWFRRGEDGRFLWPGFGDNSRVLKWVIDRIEGHVGADETVVGHTAKAEDLDLDGLDTPIEDVKEALTAPAEQWANDVEDNAEYLTFLGPRVPAEVHSQFDALKARISAAHA

SEQ ID NO: 2 - DNA, 1833 bp, Unknown
  Phosphoenolpyruvate carboxykinase NT
atgactactgctgcaatcaggggccttcagggcgaggcgccgaccaagaataaggaactgctgaactggatcgcagacgccgtcgagctcttccagcctgaggctgttgtgttcgttgatggatcccaggctgagtgggatcgcatggcggaggatcttgttgaagccggtaccctcatcaagctcaacgaggaaaagcgtccgaacagctacctagctcgttccaacccatctgacgttgcgcgcgttgagtcccgcaccttcatctgctccgagaaggaagaagatgctggcccaaccaacaactgggctccaccacaggcaatgaaggacgaaatgtccaagcattacgctggttccatgaaggggcgcaccatgtacgtcgtgcctttctgcatgggtccaatcagcgatccggaccctaagcttggtgtgcagctcactgactccgagtacgttgtcatgtccatgcgcatcatgacccgcatgggtattgaagcgctggacaagatcggcgcgaacggcagcttcgtcaggtgcctccactccgttggtgctcctttggagccaggccaggaagacgttgcatggccttgcaacgacaccaagtacatcacccagttcccagagaccaaggaaatttggtcctacggttccggctacggcggaaacgcaatcctggcaaagaagtgctacgcactgcgtatcgcatctgtcatggctcgcgaagaaggatggatggctgagcacatgctcatcctgaagctgatcaacccagagggcaaggcgtaccacatcgcagcagcattcccatctgcttgtggcaagaccaacctcgccatgatcactccaaccatcccaggctggaccgctcaggttgttggcgacgacatcgcttggctgaagctgcgcgaggacggcctctacgcagttaacccagaaaatggtttcttcggtgttgctccaggcaccaactacgcatccaacccaatcgcgatgaagaccatggaaccaggcaacaccctgttcaccaacgtggcactcaccgacgacggcgacatctggtgggaaggcatggacggcgacgccccagctcacctcattgactggatgggcaacgactggaccccagagtccgacgaaaacgctgctcaccctaactcccgttactgcgtagcaatcgaccagtccccagcagcagcacctgagttcaacgactgggaaggcgtcaagatcgacgcaatcctcttcggtggacgtcgcgcagacaccgtcccactggttacccagacctacgactgggagcacggcaccatggttggtgcactgctcgcatccggtcagaccgcagcttccgcagaagcaaaggtcggcacactccgccacgacccaatggcaatgctcccattcattggctacaacgctggtgaatacctgcagaactggattgacatgggtaacaagggtggcgacaagatgccatccatcttcctggtcaactggttccgccgtggcgaagatggacgcttcctgtggcctggcttcggcgacaactctcgcgttctgaagtgggtcatcgaccgcatcgaaggccacgttggcgcagacgagaccgttgttggacacaccgctaaggccgaagacctcgacctcgacggcctcgacaccccaattgaggatgtcaaggaagcactgaccgctcctgcagagcagtgggcaaacgacgttgaagacaacgccgagtacctcactttcctcggaccacgtgttcctgcagaggttcacagccagttcgatgctctgaaggcccgcatttcagcagctcacgcttaa

SEQ ID NO: 3 - DNA, 43 bp, Artificial Sequence
  primer 1
ggggatcctctagagtcgacctgcgacgactggaaaaccatgg

SEQ ID NO: 4 - DNA, 47 bp, Artificial Sequence
  primer 2
gcagttcttaagcgtgaactactagttaaaactttaggtgagacaac

SEQ ID NO: 5 - DNA, 47 bp, Artificial Sequence
  primer 3
gttgtctcacctaaagttttaactagtagttcacgcttaagaactgc

SEQ ID NO: 6 - DNA, 42 bp, Artificial Sequence
  primer 4
gcttgcatgcctgcaggtcgacggctggaccctagaattcgg

SEQ ID NO: 7 - DNA, 42 bp, Artificial Sequence
  primer 5
ggggatcctctagagtcgacgtggcgtttgaaaccccggaag

SEQ ID NO: 8 - DNA, 41 bp, Artificial Sequence
  primer 6
catcgagccacacgctccagtgaacaaggacctctacgaac

SEQ ID NO: 9 - DNA, 41 bp, Artificial Sequence
  primer 7
gttcgtagaggtccttgttcactggagcgtgtggctcgatg

SEQ ID NO: 10 - DNA, 44 bp, Artificial Sequence
  primer 8
gcttgcatgcctgcaggtcgacttagcagtcgaagtacaattcg

SEQ ID NO: 11 - protein, 477 aa, Artificial Sequence
  glnA(D401N) AA
VAFETPEEIVKFIKDENVEFVDVRFTDLPGTEQHFSIPAASFDADTIEEGLAFDGSSIRGFTTIDESDMNLLPDLGTATLDPFRKAKTLNVKFFVHDPFTREAFSRDPRNVARKAEQYLASTGIADTCNFGAEAEFYLFDSVRYSTEMNSGFYEVDTEEGWWNRGKETNLDGTPNLGAKNRVKGGYFPVAPYDQTVDVRDDMVRNLAASGFALERFHHEVGGGQQEINYRFNTMLHAADDIQTFKYIIKNTARLHGKAATFMPKPLAGDNGSGMHAHQSLWKDGKPLFHDESGYAGLSDIARYYIGGILHHAGAVLAFTNATLNSYHRLVPGFEAPINLVYSQRNRSAAVRIPITGSNPKAKRIEFRAPDPSGNPYLGFAAMMMAGLDGIKNRIEPHAPVNKDLYELPPEEAASIPQAPTSLEASLKALQEDTDFLTESDVFTEDLIEAYIQYKYDNEISPVRLRPTPQEFELYFDC

SEQ ID NO: 12 - DNA, 1434 bp, Artificial Sequence
  glnA(D401N) NT
gtggcgtttgaaaccccggaagaaattgtcaagttcatcaaggatgaaaacgtcgagttcgttgacgttcgattcaccgaccttcccggcaccgagcagcacttcagcatcccagctgccagcttcgatgcagatacaatcgaagaaggtctcgcattcgacggatcctcgatccgtggcttcaccacgatcgacgaatctgacatgaatctcctgccagacctcggaacggccacccttgatccattccgcaaggcaaagaccctgaacgttaagttcttcgttcacgatcctttcacccgcgaggcattctcccgcgacccacgcaacgtggcacgcaaggcagagcagtacctggcatccaccggcattgcagacacctgcaacttcggcgccgaggctgagttctacctcttcgactccgttcgctactccaccgagatgaactccggcttctacgaagtagataccgaagaaggctggtggaaccgtggcaaggaaaccaacctcgacggcaccccaaacctgggcgcaaagaaccgcgtcaagggtggctacttcccagtagcaccatacgaccaaaccgttgacgtgcgcgatgacatggttcgcaacctcgcagcttccggcttcgctcttgagcgtttccaccacgaagtcggtggcggacagcaggaaatcaactaccgcttcaacaccatgctccacgcggcagatgatatccagaccttcaagtacatcatcaagaacaccgctcgcctccacggcaaggctgcaaccttcatgcctaagccactggctggcgacaacggttccggcatgcacgctcaccagtccctctggaaggacggcaagccactcttccacgatgagtccggctacgcaggcctgtccgacatcgcccgctactacatcggcggcatcctgcaccacgcaggcgctgttctggcgttcaccaacgcaaccctgaactcctaccaccgtctggttccaggcttcgaggctccaatcaacctggtgtactcacagcgcaaccgttccgctgctgtccgtatcccaatcaccggatccaacccgaaggcaaagcgcatcgaattccgcgctccagacccatcaggcaacccatacctgggctttgcagcgatgatgatggccggcctcgacggcatcaagaaccgcatcgagccacacgctccagtgaacaaggacctctacgaactaccaccagaggaagctgcatccattccacaggcaccaacctccctggaagcatccctgaaggcactgcaggaagacaccgacttcctcaccgagtctgacgtcttcaccgaggatctcatcgaggcgtacatccagtacaagtacgacaacgagatctccccagttcgcctgcgcccaaccccgcaggaattcgaattgtacttcgactgctaa